European Patent Application EP 4 729 604 A1, published April 22, 2026. Title: 一种产D-泛酸的基因工程菌、构建方法及应用. Applicant: 浙江工业大学. The sequence listing filed with the application follows.

SEQUENCE LISTING (10 sequences)

SEQ ID NO: 1 - DNA, 1901 bp, Escherichia coli
  source 1..1901: mol_type = genomic DNA
ttgacaattaatcatccggctcgtataatgtttcacacaggaaacagaccatgcctaagtaccgttccgccaccaccactcatggtcgtaatatggcgggtgctcgtgcgctgtggcgcgccaccggaatgaccgacgccgatttcggtaagccgattatcgcggttgtgaactcgttcacccaatttgtaccgggtcacgtccatctgcgcgatctcggtaaactggtcgccgaacaaattgaagcggctggcggcgttgccaaagagttcaacaccattgcggtggatgatgggattgccatgggccacggggggatgctttattcactgccatctcgcgaactgatcgctgattccgttgagtatatggtcaacgcccactgcgccgacgccatggtctgcatctctaactgcgacaaaatcaccccggggatgctgatggcttccctgcgcctgaatattccggtgatctttgtttccggcggcccgatggaggccgggaaaaccaaactttccgatcagatcatcaagctcgatctggttgatgcgatgatccagggcgcagacccgaaagtatctgactcccagagcgatcaggttgaacgttccgcgtgtccgacctgcggttcctgctccgggatgtttaccgctaactcaatgaactgcctgaccgaagcgctgggcctgtcgcagccgggcaacggctcgctgctggcaacccacgccgaccgtaagcagctgttccttaatgctggtaaacgcattgttgaattgaccaaacgttattacgagcaaaacgacgaaagtgcactgccgcgtaatatcgccagtaaggcggcgtttgaaaacgccatgacgctggatatcgcgatgggtggatcgactaacaccgtacttcacctgctggcggcggcgcaggaagcggaaatcgacttcaccatgagtgatatcgataagctttcccgcaaggttccacagctgtgtaaagttgcgccgagcacccagaaataccatatggaagatgttcaccgtgctggtggtgttatcggtattctcggcgaactggatcgcgcggggttactgaaccgtgatgtgaaaaacgtacttggcctgacgttgccgcaaacgctggaacaatacgacgttatgctgacccaggatgacgcggtaaaaaatatgttccgcgcaggtcctgcaggcattcgtaccacacaggcattctcgcaagattgccgttgggatacgctggacgacgatcgcgccaatggctgtatccgctcgctggaacacgcctacagcaaagacggcggcctggcggtgctctacggtaactttgcggaaaacggctgcatcgtgaaaacggcaggcgtcgatgacagcatcctcaaattcaccggcccggcgaaagtgtacgaaagccaggacgatgcggtagaagcgattctcggcggtaaagttgtcgccggagatgtggtagtaattcgctatgaaggcccgaaaggcggtccggggatgcaggaaatgctctacccaaccagcttcctgaaatcaatgggtctcggcaaagcctgtgcgctgatcaccgacggtcgtttctctggtggcacctctggtctttccatcggccacgtctcaccggaagcggcaagcggcggcagcattggcctgattgaagatggtgacctgatcgctatcgacatcccgaaccgtggcattcagttacaggtaagcgatgccgaactggcggcgcgtcgtgaagcgcaggacgctcgaggtgacaaagcctggacgccgaaaaatcgtgaacgtcaggtctcctttgccctgcgtgcttatgccagcctggcaaccagcgccgacaaaggcgcggtgcgcgataaatcgaaactggggggttaa

SEQ ID NO: 2 - DNA, 908 bp, Bacillus subtilis
  source 1..908: mol_type = genomic DNA
ttgacaattaatcatccggctcgtataatgtgtggaattgtgagcggataacaatttcacacaggaaacagaccatgaaaacaaaactggattttctaaaaatgaaggagtctgaagaaccgattgtcatgctgaccgcttatgattatccggcagctaaacttgctgaacaagcgggagttgacatgattttagtcggtgattcacttggaatggtcgtcctcggccttgattcaactgtcggtgtgacagttgcggacatgatccatcatacaaaagccgttaaaaggggtgcgccgaatacctttattgtgacagatatgccgtttatgtcttatcacctgtctaaggaagatacgctgaaaaatgcagcggctatcgttcaggaaagcggagctgacgcactgaagcttgagggcggagaaggcgtgtttgaatccattcgcgcattgacgcttggaggcattccagtagtcagtcacttaggtttgacaccgcagtcagtcggcgtactgggcggctataaagtacagggcaaagacgaacaaagcgccaaaaaattaatagaagacagtataaaatgcgaagaagcaggagctatgatgcttgtgctggaatgtgtgccggcagaactcacagccaaaattgccgagacgctaagcataccggtcattggaatcggggctggtgtgaaagcggacggacaagttctcgtttatcatgatattatcggccacggtgttgagagaacacctaaatttgtaaagcaatatacgcgcattgatgaaaccatcgaaacagcaatcagcggatatgttcaggatgtaagacatcgtgctttccctgaacaaaagcattcctttcaaatgaaccagacagtgcttgacggcttgtacgggggaaaataa

SEQ ID NO: 3 - DNA, 890 bp, Corynebacterium glutamicum
  source 1..890: mol_type = genomic DNA
ttgacaattaatcatccggctcgtataatgtttcacacaggaaacagaccatgcaggtagcaaccacaaagcaggcgcttatcgacgccctcctccaccacaaatccgtcgggctcgtccccaccatgggtgcgctacacagcggacacgcctcgttggttaaagcagcacgcgctgaaaacgacactgttgtagccagtatttttgtcaatcccctgcagtttgaagcactcggtgattgcgatgattaccgcaactatccccgccaactcgacgccgatttagcactgcttgaagaggcaggtgtggatattgtgttcgcacccgatgtggaggaaatgtaccccggtggcttgccactagtgtgggcgcgcaccggttccatcggaacaaaattggagggtgccagcaggcctggccatttcgatggtgtggctaccgtggtggcgaagctgttcaatttggtgcgccctgatcgtgcatattttggacaaaaagatgctcagcaggttgcggtgattcggcgattggttgccgatctagacattcccgtggagattcgtcccgttccgattattcgtggcgccgatggcttagccgaatccagccgcaatcaacgtctttctgcggatcagcgagcgcaagctctggtgctgccgcaggtgttgagtgggttgcagcgtcgaaaagcagctggtgaagcgctagatatccaaggtgcgcgcgacaccttggccagcgccgacggcgtgcgcttggatcacctggaaattgtcgatccagccaccctcgaaccattagaaatcgacggcctgctcacccaaccagcgttggtggtcggcgcgattttcgtggggccggtgcggttgatcgacaatatcgagctctaa

SEQ ID NO: 4 - DNA, 1763 bp, Bacillus subtilis
  source 1..1763: mol_type = genomic DNA
ttgacaattaatcatccggctcgtataatgtttcacacaggaaacagaccttgacaaaagcaacaaaagaacaaaaatcccttgtgaaaaacagaggggcggagcttgttgttgattgcttagtggagcaaggtgtcacacatgtatttggcattccaggtgcaaaaattgatgcggtatttgacgctttacaagataaaggacctgaaattatcgttgcccggcacgaacaaaacgcagcattcatggcccaagcagtcggccgtttaactggaaaaccgggagtcgtgttagtcacatcaggaccgggtgcctctaacttggcaacaggcctgctgacagcgaacactgaaggagaccctgtcgttgcgcttgctggaaacgtgatccgtgcagatcgtttaaaacggacacatcaatctttggataatgcggcgctattccagccgattacaaaatacagtgtagaagttcaagatgtaaaaaatataccggaagctgttacaaatgcatttaggatagcgtcagcagggcaggctggggccgcttttgtgagctttccgcaagatgttgtgaatgaagtcacaaatacgaaaaacgtgcgtgctgttgcagcgccaaaactcggtcctgcagcagatgatgcaatcagtgcggccatagcaaaaatccaaacagcaaaacttcctgtcgttttggtcggcatgaaaggcggaagaccggaagcaattaaagcggttcgcaagcttttgaaaaaggttcagcttccatttgttgaaacatatcaagctgccggtaccctttctagagatttagaggatcaatattttggccgtatcggtttgttccgcaaccagcctggcgatttactgctagagcaggcagatgttgttctgacgatcggctatgacccgattgaatatgatccgaaattctggaatatcaatggagaccggacaattatccatttagacgagattatcgctgacattgatcatgcttaccagcctgatcttgaattgatcggtgacattccgtccacgatcaatcatatcgaacacgatgctgtgaaagtggaatttgcagagcgtgagcagaaaatcctttctgatttaaaacaatatatgcatgaaggtgagcaggtgcctgcagattggaaatcagacagagcgcaccctcttgaaatcgttaaagagttgcgtaatgcagtcgatgatcatgttacagtaacttgcgatatcggttcgcacgccatttggatgtcacgttatttccgcagctacgagccgttaacattaatgatcagtaacggtatgcaaacactcggcgttgcgcttccttgggcaatcggcgcttcattggtgaaaccgggagaaaaagtggtttctgtctctggtgacggcggtttcttattctcagcaatggaattagagacagcagttcgactaaaagcaccaattgtacacattgtatggaacgacagcacatatgacatggttgcattccagcaattgaaaaaatataaccgtacatctgcggtcgatttcggaaatatcgatatcgtgaaatatgcggaaagcttcggagcaactggcttgcgcgtagaatcaccagaccagctggcagatgttctgcgtcaaggcatgaacgctgaaggtcctgtcatcatcgatgtcccggttgactacagtgataacattaatttagcaagtgacaagcttccgaaagaattcggggaactcatgaaaacgaaagctctctag

SEQ ID NO: 5 - DNA, 891 bp, Bacillus subtilis
  source 1..891: mol_type = genomic DNA
ttgacaattaatcatccggctcgtataatgtgtggaatttcacacaggaaacagaccatgaaaacaaaactggattttctaaaaatgaaggagtctgaagaaccgattgtcatgctgaccgcttatgattatccggcagctaaacttgctgaacaagcgggagttgacatgattttagtcggtgattcacttggaatggtcgtcctcggccttgattcaactgtcggtgtgacagttgcggacatgatccatcatacaaaagccgttaaaaggggtgcgccgaatacctttattgtgacagatatgccgtttatgtcttatcacctgtctaaggaagatacgctgaaaaatgcagcggctatcgttcaggaaagcggagctgacgcactgaagcttgagggcggagaaggcgtgtttgaatccattcgcgcattgacgcttggaggcattccagtagtcagtcacttaggtttgacaccgcagtcagtcggcgtactgggcggctataaagtacagggcaaagacgaacaaagcgccaaaaaattaatagaagacagtataaaatgcgaagaagcaggagctatgatgcttgtgctggaatgtgtgccggcagaactcacagccaaaattgccgagacgctaagcataccggtcattggaatcggggctggtgtgaaagcggacggacaagttctcgtttatcatgatattatcggccacggtgttgagagaacacctaaatttgtaaagcaatatacgcgcattgatgaaaccatcgaaacagcaatcagcggatatgttcaggatgtaagacatcgtgctttccctgaacaaaagcattcctttcaaatgaaccagacagtgcttgacggcttgtacgggggaaaataa

SEQ ID NO: 6 - DNA, 918 bp, Escherichia coli
  source 1..918: mol_type = genomic DNA
gtgaacttcagacgcctgaaatactttgtaaaaattgtcgacatcggatccctgacgcaggctgctgaagtattgcatatcgcacaaccagcgctcagccagcaggttgccacactggaaggtgagttaaatcaacaacttttgatccgtacaaagcggggcgttacaccaacagacgccggaaaaattctctatacccatgcgcgggccattttacgtcagtgtgaacaggcccaactggcggtgcataacgttggtcaggcattatcggggcaagtctcgattggctttgcaccaggaaccgctgcgtcatccatcaccatgcccttattacaggcggttcgcgctgaatttccggagatcgttatctatcttcatgaaaatagtggtgcagtgcttaacgaaaaattgataaatcaccaactcgatatggcggtgatttatgagcattcccctgtggctggtgtatccagtcaggctttgctgaaagaagatctttttctggtaggaactcaagattgcccggggcaaagcgttgatgtgaatgctattgcgcaaatgaacctctttctccccagtgattacagtgctattagacttcgtgttgatgaggctttttccctacggcgactcacggcaaaagttattggtgaaattgagtctattgccacgcttaccgcagcgattgccagcggcatgggcgttgcagtattacccgaatcggccgcgcgttcgttatgtggcgcagtaaatgggtggatgtcacgcattaccactccttccatgagtctctctttgtcattaaatttacccgccagagcgaacttatcgccacaggcacaggcagtgaaagagttgttaatgtcagtgattagttctccagtgatggaaaaaaggcagtggcaattggtgagctaa

SEQ ID NO: 7 - DNA, 102 bp, Escherichia coli
  source 1..102: mol_type = other DNA
tgcttcaaactttcgcccctcctggcattgattcagcctgtcggaactggtatttaaccagactaattattttgatgcgcgaaattaatcgttacaggaaaa

SEQ ID NO: 8 - DNA, 1284 bp, Escherichia coli
  source 1..1284: mol_type = other DNA
gtggctgatacaaaagcaaaactcaccctcaacggggatacagctgttgaactggatgtgctgaaaggcacgctgggtcaagatgttattgatatccgtactctcggttcaaaaggtgtgttcacctttgacccaggcttcacttcaaccgcatcctgcgaatctaaaattacttttattgatggtgatgaaggtattttgctgcaccgtggctttccgattgatcagctggcgaccgattctaactacctggaagtttgttacatcctgctgaatggtgaaaaaccgactcaggaacagtatgacgaatttaaaactacggtgacccgtcataccatgatccacgagcagattacccgtctgttccatgctttccgtcgcgactcgcatccaatggcagtcatgtgtggtattaccggcgcgctggcggcgttctatcacgactcgctggatgttaacaatcctcgtcaccgtgaaattgccgcgttccgcctgctgtcgaaaatgccgaccatggccgcgatgtgttacaagtattccattggtcagccatttgtttacccgcgcaacgatctctcctacgccggtaacttcctgaatatgatgttctccacgccgtgcgaaccgtatgaagttaatccgattctggaacgtgctatggaccgtattctgatcctgcacgctgaccatgaacagaacgcctctacctccaccgtgcgtaccgctggctcttcgggtgcgaacccgtttgcctgtatcgcagcaggtattgcttcactgtggggacctgcgcacggcggtgctaacgaagcggcgctgaaaatgctggaagaaatcagctccgttaaacacattccggaatttgttcgtcgtgcgaaagacaaaaatgattctttccgcctgatgggcttcggtcaccgcgtgtacaaaaattacgacccgcgcgccaccgtaatgcgtgaaacctgccatgaagtgctgaaagagctgggcacgaaggatgacctgctggaagtggctatggagctggaaaacatcgcgctgaacgacccgtactttatcgagaagaaactgtacccgaacgtcgatttctactctggtatcatcctgaaagcgatgggtattccgtcttccatgttcaccgtcattttcgcaatggcacgtaccgttggctggatcgcccactggagcgaaatgcacagtgacggtatgaagattgcccgtccgcgtcagctgtatacaggatatgaaaaacgcgactttaaaagcgatatcaagcgttaa

SEQ ID NO: 9 - DNA, 1284 bp, Escherichia coli
  source 1..1284: mol_type = other DNA
ttggctgatacaaaagcaaaactcaccctcaacggggatacagctgttgaactggatgtgctgaaaggcacgctgggtcaagatgttattgatatccgtactctcggttcaaaaggtgtgttcacctttgacccaggcttcacttcaaccgcatcctgcgaatctaaaattacttttattgatggtgatgaaggtattttgctgcaccgtggctttccgattgatcagctggcgaccgattctaactacctggaagtttgttacatcctgctgaatggtgaaaaaccgactcaggaacagtatgacgaatttaaaactacggtgacccgtcataccatgatccacgagcagattacccgtctgttccatgctttccgtcgcgactcgcatccaatggcagtcatgtgtggtattaccggcgcgctggcggcgttctatcacgactcgctggatgttaacaatcctcgtcaccgtgaaattgccgcgttccgcctgctgtcgaaaatgccgaccatggccgcgatgtgttacaagtattccattggtcagccatttgtttacccgcgcaacgatctctcctacgccggtaacttcctgaatatgatgttctccacgccgtgcgaaccgtatgaagttaatccgattctggaacgtgctatggaccgtattctgatcctgcacgctgaccatgaacagaacgcctctacctccaccgtgcgtaccgctggctcttcgggtgcgaacccgtttgcctgtatcgcagcaggtattgcttcactgtggggacctgcgcacggcggtgctaacgaagcggcgctgaaaatgctggaagaaatcagctccgttaaacacattccggaatttgttcgtcgtgcgaaagacaaaaatgattctttccgcctgatgggcttcggtcaccgcgtgtacaaaaattacgacccgcgcgccaccgtaatgcgtgaaacctgccatgaagtgctgaaagagctgggcacgaaggatgacctgctggaagtggctatggagctggaaaacatcgcgctgaacgacccgtactttatcgagaagaaactgtacccgaacgtcgatttctactctggtatcatcctgaaagcgatgggtattccgtcttccatgttcaccgtcattttcgcaatggcacgtaccgttggctggatcgcccactggagcgaaatgcacagtgacggtatgaagattgcccgtccgcgtcagctgtatacaggatatgaaaaacgcgactttaaaagcgatatcaagcgttaa

SEQ ID NO: 10 - DNA, 78 bp, Escherichia coli
  source 1..78: mol_type = other DNA
tccaataaatcatattgttaatttcttcactttccgctgattcggtgccagactgaaatcagcctataggaggaaatg